European Patent Application EP 4 151 734 A1, published March 22, 2023. Title: Polynucleotide from Human Genome and Method of Preparing a Polypeptide of Interest Using the Same. Applicant: SAMSUNG BIOEPIS CO., LTD. The sequence listing filed with the application follows.

SEQUENCE LISTING (48 sequences)

SEQ ID NO: 1 - DNA, 3430 bp, Artificial Sequence
  Synthetic: CCE1
ctcccctactgagctcccagtatgttccaggccctgtgccagggccttcacctccattatcttacttaaccctcacatggatcctaagttaggggttattgcgccatttcacagaaagagtctgaagttcagaggcccagtaacctgcctaagagagtaagggaattcagattaaggtcttttgactttatgctgtctcttgctagtccagattctactgtcagggactgtggactccaggaagctgccttacagtttgtgcttgtcctggctctttctggcagctctcttctgatggtcatcctgtgtccatcattgtgtccccatatgcagtgctggtgaccattttgctcaatcttttgacccggaagcctgaaagagcagtgttaactacctgctatgatacaagcactgtgccttggttattgtttgatggatgcagtaactggaaaacagccatttaactgtcagaaaataaagattgaagctctattttgaattttagtacttattttcaaatagctacacatttaagatggtaagcatcattcttttcattgaatacttaatctcatcgaatgaaaagatgaaaaatagaaatatatatcattaaaccatcctctcacatactttaacctttcagagaatacatattttcaaccaaggtagacaacaatgttaaggcaaaaaagtagtgggttggttaaagtttagtttatttgatctgaatgagtgcctttttgctagtgttttccaatacatcatatcatttctggaatgagaagtactcattgtagtagatgtttttatgattatcaggaaactgtattagggaaaagcaggaagatatttagttcaatattccagataagatgattaataaattgtatactaaaagtaactctacttattttaaaatatcttaactctcactgtttttctccacttctaggggaaaagtgggtgtttccccaatgtgatagtgtattgggttaataatacaaattgtatttgtgacattttctgcattgctttttgacaacttcagctttcataatctaatacagtcaatattcgtttttgtaaataacactgaagtgaaaaggaagattgccattttctagataaaccaatcaataatctttgtggcccagattgcttcagctcttaaattttcccaatgcgaaaccttaaagaatgtttaaattgtttaaacactgtcaacagtctgtggcacatctagtcccagcttactctaggatggtttttactattcaccaaggaactactcgttacctttgttagattgtgtttacagtgcaagttttagcaagacagtgtatagttccaagcctgagcctctcagatggatactgaggatacaccttagtggtgtttcctctatctgatcccttccttttctgagactatgcctatctactacgttcatagaggattcacatcgatatgctaaattcactcattgcttaatatttatatttatgtatttgataaatatataagtatttacagagcaaaatctactctgtaccagatattgttccaagctgcagatagagtggtgaacaaatgatcaaaatttctgccctcatggtccttctaatctaaagagagaagacaagtaaacaagaacagtaaataaatattagctaacatttttgcctgtatccttcatggatcttgtgaatagaatccctcttctaattctggtttagaagatcctgattcttatataataggttcctgactggtttctacagtgagcagcttttatgaattttgtgaatttgacatgcttttattggggagattatatctgatctgtgaaattaacataaattaatcatatcattgtgaaccttaaaggtagattcttaaatggcatcagctagatatttttacacttgatcttagccaaaaagccaagaagcagtagctagatatgtttaaaacattctctttatcggttgcacatggtggctcatgcctgtaatcccagcactttgagaggctgaggcaggaggattgcttgagcccaggagtttgaaactagcccgggcaacatagtgaggcccccattgctacacaaaaatttaaaatataattttaaaaataaataaaataaaacattctctttatcagttcttctcttctgcatggcataaaggaagcagctggacctgaatgccaagtggattgattcattacttgcattagtaaataagatgctccatcattatgagtgtgtttcattgagttgtggagatcttttgttaaattttgcaatgctgtgtcttgcagaaaaaatgaaaatgttggattccattttttttttttttgctttccatgagtttcctgcacatcataatgcaggtagggtgaggggtatggagagggagaacccagccagaaatggagcaaggcattttgcagaggctacttcaaaggagaaattgacaattacatgcattctcacgttcttcctgcttttcacgtcctctctaaataaaagtagagactataaatatataccacccatttgtttttagagagtggtgtgataaagatttatttaaaacaacataggctttgctgacagtaacagctcagcaagaatttttttttttctttttgtattggttctattcttcccacagccctttactccaggtttctatgccaacgactgaaatcaaaggcttttcacaatgtgtatgttctggaatactaagtaaattttgttgttgctaagagggaaacttggttttagccagcaggccatgtagaaagcagagtttgtcttaatgcttaccagatataacccctcacttctaatagaatttgacccatggcttataatagaatttcttttggatatgcgacatttcattttaagtttcttttagtaccttgtccatactaactcacagaagatatttcttttatcttcaaagaaagatacattttcactttcaacctctctcagaaggaaactcaagaagcggaaagtgtgaagtctttgtagggatgttgcttgttgtatatttgcctcctttcttttaaacacctaaattcatccctcctgatgccatgctattaatattgccttccacctgtaatgtacctatacatgttttacctcacttgagcttcccaatggtcctcagagtaaaaagcattatttttcccaactcagagagcgtaggagccaaagtgtggctttccagctctaagcccagtgttctgtgggttacatcaccttgttttttattccaaagttaacttgtgaacccttctaataaactgctccaagatatgacaaaatcactttatcccaacaggctctgaagttgtaagatgcccctttggaaacagggactcctgtggatatgggggtggtcgttcatgg

SEQ ID NO: 2 - DNA, 3730 bp, Artificial Sequence
  Synthetic: CCE2
ttgtgtgggtctatttctaggttctctactctgtttcattgatctgtgtgtctgtccctccaccaatactacatagtcttgattattgtagctacataataagtcctgaaattggatagagtgattcctcccactttattctcccttttcaaaattgttttggctattctagtttctttgcctttccatataaattttggaataaacttgtctatgtttaaaatatcctcctggaattttgatagagattgagctaaaactatacataaatttggggagaactaacatctttactatgttaagtcttctgatccatgaatgtggcatatttctttctctatttaggtcttctttgatttctgtcatcagcattttgtagttttcagcatataagctctatacatatcttgttacatttacacttaagtattttgttcttgagcaagtgtaaatggcactgtatttttaatttcagcatccatgtgttcattgctagtatatagaaatacaatttatttttgcaagcttatcttgtatcctgcaaccttgctaagctcacttattagttctaggaattgtcttgtagattccttgggattttctatgtagactataatgccgtctccaaataggagcagttttatttattcttttataatctacatgttttatcttttcttttttcttctttttttttttttgccttattacactggttagaacttccaacactatgttgaattaaggtggtgagagcagagatccttgccttgtttccaatctgagggggaaagcatttagtctttcaagcattgtgtttaatgttaggtataagtctaatattgcttgatccagaaaaaaatatatatatatttggtgtaagttgtatgtagatgctcaagttaaggaagttccctttttgccctatttctcagagttttttttaacttataataagtgttagattttatcaaatgctttttctgcattgattaatatgatcatgtgatttctattagtttgttacactgattgtgtagaattagcatacaattctttaaacatttggtagaattctccagtgaaaccatctggacctggagattttaaagggagtagttttaaaattatgaatttcatgtttttaatagttatagggctattcaaatcatctatttcatatttggtagatttgggaagtttatatttttcaagaaattggtctgtttcatcaaagttgtcaaagcatgtagcattgttcatagtattcccttattacccatttgatgtctgaaggctctgtagtgatattcatttccttcctgatatgagcaatttgtatgtcttgctagaggtttgtcaatcttactgatcttttcaaagaagcagctctttatttcattgattttctctatttttctattttcaattctgcttatttatgctgttatttttattattttcttccttctgtttgctttggctttattttgctctccttgttctagttacttgaggtaggaacttagatgattgatttgagaccttttttcttttatagtataagcatttggagctataaacttctttttaagcattgctttagttgcatctcataaatttttctatgttgtattttcattttgattcagttcaatgtatttttaaaatttatcttgaaatttaaattttcatatttgacccatgggttattttaaagtgtgttgtttatttttcaagttttagatattttcttatctttctgttattgatttccaatttggtcacagaatacatttcatttgatttcaattattttaaatttgttgacatttgttttatgacacaggatatgtctaacatgttttgtattccatgggcacttgaaaaggatgtgtactcttctgctgttggatgagatgttctataaatgtcaaatcaaatcctgttgtttgagggtgttgttgagttcctatatacccttgctgattttctatctagtaggtctatcccagatgcctgctcagccttctctgacttcaccccagtggggaaatttggggcacctggttatagcttagcaagggtgaaaagctatgttttcaacccctcctttgctggtggggttgggaacgggaccacatatttttttctgtggtatttggctaaagaattagtgtataaaaatttctgtcttggtaagagagcatgatttttaaaaaatctgcccctgttggtattttcagtttgcagactttttcagcttcaactctgggatatatgaggcaaaacaaaaatccagggaactcaccacatgccgttccttgagtcctgaggtctcttgcaggtgtacattcttctctccacctcctctccagtctttttgtgttcattttatatataatgctcacggttttttgttgtgctttagagggaggaccagggaaaagtatgtcattccatcttcccagaagcagaagtcctaacttattcttttaaaatgttatgtaactttgcagagtatgacttttatcaggatttatttaactattcacccattgatgaacttttaggttgtttcttaattgtggtggctaacacaatctttcaataaacatccattcaataaacatttgtgtacacgtgcaggagtttcttcatgatagatgctaagtggcgttgctgggtaataggggatgcacattttccatgttaatgggtgttgtccaatttctacccataatggctgtgctccacccagcagtgtatgagagtagcagttttgctcaacttcttgacaacacttgataatagtcagactttgagttccgaatgtaatgagtgaaagatgatatctggtggttgttatcatttgcctttccttgattcccagaggctgaatatcttttcaaatgtctgttggccatctgtaactctccttttgaattacctgtccatatactttgcccatatttattttgagttgtttacctttttattgatttacagaaattctctatatatttttattgttctttgtctaatacatacatttcaaatatatttccccagtttattatttgtcttttaactttattgatggtgtcttttgcctaaaaaaaaattattcttttgtgtagattcaaatttgtcaaccactccctcctggcttttgggttgtgtttgtgtgttgtttaaaatgactttctccataccaaagtcacaaatatataaatctctatttttcccattacaggtttctattcttttttatatttagttgtttgagctatgtggaatatgtgtgtgtatagtatgaggtagggatctcatttaatttttatcaaatggaaagctagttacttcagcactattcgttgaatagtccattctttcaccactgacttataaatgcagcttttattattttatttaacacctttacatgagttggcttgagagctctctgttctctttcactcatttgtctacttctgtgccaatgccacaccctgttaattactgtagatttgataccttgtataatgtcatccttcatttgttcttttccccaaaaaaattgttttggctcttcttatacatattctttttcacatggattttagaatcagtttgtcaggttctgtgaaaaattcctctggagatttgattgaaatagcaatgagattatagattaatttagggagacatcttttctccttttctccac

SEQ ID NO: 3 - DNA, 3000 bp, Artificial Sequence
  Synthetic: CCE3
tattggcatcttaacaatattaaatcttttgcaccatgaacatggaacatgtttccatttatttaggtcttctttagtttctttgcatgatgttttgtacttttcagaatagaagttttgcatctcttttgttaaatttatttctaagtaatttactctttttgatactattgtaaactgaagtgttttcttaattttattttcagattgttactataacattttgaataagatacaaaaaatcaccatgatcaatcaaagtttaaaatcaaaggttgttaatatatatttttaggttgttgtttcagggcttcctgtgttttacaatgtccagcacagtaacaaggctttaaaaaattatcacattagtatgttttggtaatgtggaaacaattgacctcactaatggatttaagattatcataaaaattctaagccaatactatcatatctgagaaaagttaatgtgaaactgtttactttggttgttccagaaacctgtcttctaatagttaaagtatttaatatgctccttgggtgactggctatttccataattatagttctttctctaaaaaacgtggaaaattcttgggtgttggcattaaatgtcttgttttctttaatgaactgaaaatcagatccaatcagattaaaattttctcaaggaccaagatctggactctgcagttaatgttctggatgagttttgttttttgcagtagacataaattcacaccaactcctcacctagagaagtcagtccctccgtttctctatttttcccttaagacatcacacttagcatagtcctctctctttgaattgctggttctccttgctttatgcctaattaaataataaacaactttatcaaaatatctagtatgttattggccagaaatcaagtatacagtgaacatttattttacttgaaacaatattttttatcttaaaaaaggtttttatgctagtcagggttttagaatgtttacccagatgttgtgtcaacttttaaaaagaaatttcatagacgggaggcatttgagaagttggaaaggaccttagaaatccagcacaggggtctgtgagccaagttcagcctgtaggcatgttttacttggccctggtggtattttaaaactatttaaattagttgccaacatttacaagtcataaaaatctggatttctgccttttcttgaaaaagtgggtaaacctggccatctcagggctacactgcagcatggcacatactgggtgcatatgcactccatccagtttctcagggtcctcctgtaggctcacttccatcagttgcatgacctgctgaccctgggggaggcccctttgcatctgtgactcctgagctaacgtaatccccttctgaggttttgagactgaggtttggaaaaatcattactgcccaaagctagtcaacagctaatcagttgtcaatttcttttcttttctttttttaatatttatttatttatttatttatttatttatttatttattaattatgtatttatttattcattcatttattcatttattttgagatagggtctcactctgttgcccaggctggagtgcagtggtgctgttacagctcattgcagcctcgacctccccaggctctggtgatcctcccacttcagcctcctgagtagctgggactacaggcatgtgccactatgcctggctaatttgtgtgtgtgtgtgtgtggcgaaagggtttcgtttctccctgttacccaggctggttgcaaactcctgggctcaagccatccatctgcctcagcctctcagtgctgggaatataggcataagccaccttgcccggcctagttgtcaatttcttaataatgccaagagtattatttataaaacagataaagttagaggagggctaattattctacattttcaaaggactttcttgcttgaatggcatccccattgatgtagttaggcttttaaaatataatgaactgacggaggatccagggaagagccacagcaaatcagagtgattatacctaaaaacaataaaatgtgttctgaatcatcatcgtttcaatctatctcccagtttatatctgacctcctctttaaaattttctttcttgtctttcttttgtttctctcctcttcttccaaaccctatgatttatttatgtatctgggtcacaactaagttagtccttaatcatctgttcattcattaaatatttatttcaacacttactagctgccaggtgctgttctggtcacttgggatagcacagtgaacaaaagggacaaaaattccttgcgccacttacatgctagtgggagaatgagatgataagtaaacaaagaagatcatttctgatagttataggcactccgaaggtgtaaaaacaggacaatgtgacagctggggttggggtctatgaagccagccatatcaaagtgtggggaagagtgatgtaggctgagaggaaaacaagcacaatggccctgaaatggaaacaagcttcgtgtgttcaatgaagggacaggctaattggtaggagctgagatgggggaggggggcaagggacaggcatgcagggccttgcaggccatggacataggtttagattttattccgcattaggagcccttggaggggtttcctttatattggccatgacttatacagttgtctcgctcttgatatccatgggagattggttccaggaccactcactggtgaacaccaaaatccacaggtataatccctgatagaaaatgttgcagtattcacatatcacctatgcacatcctgccgtatactttaaatcatctctagattacttatcacacttattacaatgcaaatgttatgtaaaaggttattatattgcatttttaaattttgtattttttttgttgtattattatcttttactgtgaggtttttaaagaatttttctgccagatgtgctggctcacatctgtaatcccagc

SEQ ID NO: 4 - DNA, 3298 bp, Artificial Sequence
  Synthetic: CCE4
ttttgggcagagattagttgggggatgtgggtgggaaacctggtgattagatatatttaaacgtgtcatgtcagtatagagcgtgaattaaaaataaattatatttggagagttgtaagaaatttaccagtcccttcagacagacacatgaccctttaaaactcattaaaactccttggcacaatggaataacatgcactttggtcttggaagaaaccattaggttgcaatgtttttgatttctctaccactgacttgctctttgatcttggaaagtgactgacttgtcctgtgattgtttcataatcacccataataaaactgacttactgtatatagtgaatagttaagtttaaaactatatctagtttccgttatagctcaagtttatgtattattttattagcgtttagatgttaacattaagctttcaaatcagatgaaatttaatttgaaaaaagttttcgtgtatgaatactttatattctgcagttcatacatgcagtaccacccttaattaaatgatatttccacaaatcagtttggaagattttcttcctgcaaaatgtatgtttaaaatacataaaaattgatgggaccatgtacttatggctagtcggaaagtggaaagttttttagatttatgcttaggacaggtgatagtacttgagcttctattcttagtttgaccttgcctcccccacccccttaaagcaagacacttaatctctttaatgtctcagtttattcatctttaacacctgtattcttatttcatgaaaacgatacctggtttatatttggtagcatttaaggacttgatatagaaggtggtatggaagttcaaattatatagaaagtatttgtatgctgaatgataatcttgacaaattactgattactacatttagaaagttacaactctggagggaattgatatttgatattgttttcctgtgtgttctaagttaccaccataacagtaggaaaataaaccctatcctggctgtgttacaaagggattaactcacttcttcaagttgttactaaatctccagccctttaaacaacagaaataaaaagtgttccttattttaatttttccgaaatgaaagtcctataactaaccttggcttaattttttcttttgttgagggctttccaagttattttctttgtgaggaatggaggctaaaccatgtcagttgcttgaagcaactaaaaataccccgtacaaatatgcagaggagtatgcttttgatttttagatcaaaacgaagaagcaagattttatggagcttgcttattatacatttattatactgagctacttgtgccttttcaaataattaaatattaactaaatacaagaggattaaatagctagactttaaataaaactaaaatagccatattagtattttctaaattctgtatcattgaaagtttaggctgatatgaaagagagggaattcctatcatggggattgccagtcttttcacaatgacctgccactagattttatagtatatgataaatgtgtgtgtgtttattgtgaaaattgtgtgagtcatatgaaaaattaagtctacttgaaaaatcaaaagacattacctacttgggtacaaagcctgatttatatatatatttctttaatgaccatattatgttatgttaaagtttgtatagtacttggacatatattatttaatttcattcctaaaacaattcaatagggaaagcaagacagatattaatattcccatttcatagatgaggaagaaaaaataacttggcttgtaagcaattcagcagagtcagagattgcatttgagatttttgattctaagtctagtgtgctttccttgggttacaacacaataaagtcaaaaacatttactgttattttcattaattgaaagcttaaaatcaatttaaaattctaacagtataaaatttaacagtataaaaatattgttaatttaattttatgacgttaatttttaaattgatttttgaatttgctaaaagtgttttaaaatcagtatcctgtttcacaattcctgaattaatctcttctctgtacatttcctgttccagtatgataatttatataggctttagcatttacttatggtattaaatgagtagacagttggaagggaattaaaattaattaggtcttgcagttcttataatactcctggtttgccacactgaattgccatgacgtggctggggatccctgttttaacatctaacaaagatagctgccagtgtacttaattttaaaacggtctcatctattaagctgctttataaacatcagccccttttctgaagtccaaagttagttttttaaaatattcactgataatggagtgggggtgctggtgacgtttctctttcttgtttatctgtaaagacagggaggtgcaatctaagttaggaaattggtgacaaatagtcatagaacatgggtcacctggcttcaattagttatgtgacctttaagaaaacaagtgcccgtttcagaaaagactgacctttgaggctagagacatcaagctactcctctacttttaggaaaaaacaatgacagggttaatttaaaactctgatgcagacagagttgaaaaatccatgacagatttatataacgaacgtggatggtgttttgttttcccagaatgcagttttaaggtcagacctatgactcagagctgtgcacttccctggtggtatgcatcagtgacatgttgccagtctaatcgtccagaagggcttgtgcccagctcggcttgctccattataatccccagctgagaagccacctttcattttttttaaatagataaggaagacagcatgaacatttgaaactcaaatactatatgtagtttataacttttcagcctgaagacttgatgcacactaagttgcctctttaattttgagaagtataatctccattgccactaatccatcatggtgtggcactgcatgaggatatgttgtgtgcattgtcagtatcggcgttttgctgagtttactgttttttagttcattggcaaggcatcgtgggttttggtgcaaagagcatggatttggaatcaaaagccacttcctctctgggtggctgattagctgagggtaaccttcacatagctggcatgggatttccagatggcatcctctctgcatgaacaaaaacaatgtgccatttcagtaaactttggtgggtgctccctcatccactccagatcttttcatctctttccttttattccctccctt

SEQ ID NO: 5 - DNA, 3341 bp, Artificial Sequence
  Synthetic: CCE5
cgcgttgctgttgttggatgaggtagtataaagatttctattatatcagttgatggtgttgttgagttcaactatgtctttactgattatttgcctactggatctgtccatttctgatagaggggtattgaaatctccaactataatagtgaatttatctatttctccttgcagttctctcaatttttacctcacatattttgaccctcttttgttagacatgtacacattaaggattgttatgtcttcttggaaaattgacccctttatcattatgtaattcctttctttatccctaataactttccttgctatgaagtttgttctgtctgaaaataatataggtactcccactttcttttgactagtgttagcacggtacatctttctccatccctttacttttaatatatatgtgtctttataaggtaaagcgggtttcttgtagataatacatatttgggtcttggtttgtgatatactctaacaatctctctcttttaattggtgtttttagaccaatgatgtttaaagtgattattgatatagttggattaatatttaccacatttgttactattttctatttgttgccctttatcttttttcctatttttgtctcccatgctttttctgacttttatggttttaattaagcatttttatgattccattttctctcctttcttggcacatcagttatacttttttaaaacagtttttagtggttgccttagagtatgcaatattgggttaacgactaatcaagtccattttcaaatagcacgataccacttcaaagtactgcaaatatcttataataactgcatagtcccaaatcttccctcctattccttgtattattgctgttatccatttaacttcttatatgtataacagaagttaataatagaatatgtatattctattaatgtcttcatatatataatagaacttcacgaacttctttatatatacaatagaacttctattatatataaaataaaatacattgttagtattattatttttaacaaactattagatcacttaagaataagaaaaataagagtatcttgctctacggactgagctagccaggcactatggaatactacacagtcataaaagagtatgaaatgatgtcctttgcagcaacatggatgcagctggaggccattatcctaagttaattaatgcagaagcaaaaaatcaaataccacatgttctcacttattagtgggagctaaacattgggtacccacagacataaagatggaaataatagacactagaaactccaaaagcaggttgggaagaagagggacaaggattgaaaaacaaactattgggtaatttcttcattactggggtgataggttcaacagaagctgtactccctgaatctaaaatacaatttattaaaaataataagaaaaacaattttttaaaattttaccttcacttattacatttctgatctatattattttcttgtctctgaggaacttattttaacatttcttgcaaggcaggtctactggctacaaattccctcaatgtttgtttaaatctttatttttcctttacttttgaaaaaaatatttcacagggtagacaattctaggttagtttttttttttttttttttttttttttttggtcctctcaacactttaaatatttcattctactctctttttgctagcttggtttttgggaagtcaggtgtaattctttattttattttatttttatttatttatttatttattttttgagacagagtctcattccgtcgcccaggctggactgcagtggcacacgatctcggctcactgcaagctccgcctcccaggttcacgtcattctcctgcctcagcctcctgagtagctgggactacaggcgcccgccaccacaccctgctaattttttgtatttttagtagagattgttagccaggaaggtctcactctcctgacctcatgatccgcctgcctcggcctcccaaagtgctgggattacaggcatgagtcaccgcgcccggcccagatgtaatttttatctttgcttctttataggtaaggtgttttttccgcatctggcttctttcagattttttttctctaactttgattttctgaaatttgaataagatatgctcaggtgtagttttttgtgggggttgggggtatttatcctgcttgttattctctgaggttcctggatctgtggtttggtgactgacattaatttggggaaattctcagtcattcctttctttcttcttattcaggtagtcgcattacatgtatgttatattttttgtagttattccacagttcttgcatattctgttctctttttttgttttcagtctttttctctgcttttcagatttggaagttagtttctttcttccttccttccttccttccttccttccttccttccttccttccttccttccttccttcttttctttctttcttttctttcctttctttccttctttctttctttcttctcttttttttatgagatggagtttcgctcttgttgcccaggttggagtgcaatggtgcgatctcagctcaccacaacctcctcctcccaagttcaagcgattctcctgcctcagcctcccgagttagctgggattacaggcatgcaccaccacgcctggccaactttgtatttttagtagagacggggtttcaccatgttggtcaggctggtctctaactcccgacctcaggtgatccacctgcctcggcctcccaaagtgctaggattacagcgatgagccacctggtgcctggcccagatttggacatttctaatgacaatcttcaacttcagggattcttcctcggttgatctagtgcactggttcatgcctataatctcagcactttgggaggctgagatgggtggatcacttgaggccaggagtttgagaccagcctgggcaacatagcaagaccccatctctacaaaaaatatatatatataaaatagctgggcatgctggtgtgtgcctgtggtcccaggtactcccgggaggtccaggctgcagtgaaccataatcaaatcactgcactccatcctgggtgacagagtgagaccctgtctaaaaaaaaagagatttttcctcagccatgtctagtctactaatgagccaatcaaaggcattctttatttctgttactgtgtttttgatttttagcattttttaattctttcttagaattttcatctctctgcttatgttatccatctttttaaaaaatttttcttttttctttttttccttaccagcagctaaaccaatatccgg

SEQ ID NO: 6 - DNA, 2152 bp, Artificial Sequence
  Synthetic: CCE6
ccgtctgttttgtttcggtttttttgagagagggtctcgctctgtcacccaggctggagtgcagtggcgcgatcatggctcactgcagcctcgacctcctgggctcaagtgatcctcccacctcagcctcccaagtataatagctgggatacaggcacacgccaccacacccagctaattcttgtattttttttgtacagacggagtttccctatgttacccaggatggtctcaaactcctgggctcaagcgattcatccacctcagcctcccaaagtgctgggtttacaggcatgagacaccacacctggccaccatctgtttttcagaataggttcttcttgtcataaggacaaagcaaagcaaaagatcatgaaacaatgttttttctttttttttttttttttgagacggagtcttgccctgttgcccaggctggagtgcaatggcgccatctcggctcactgcaacctccgcctcctgggttcaaacgaatctcctgcctccgcctcctgagtagctgggattacaggcactcgtcaccatgcccaatttttttttaaattatttttagtagacacggcgttttaccatgttggccaggttggtctcgaactcctgacctcgtgatccacctgcctctgtagaaggagggatcagactatccccaaaagaccacccctcacattcaacaagtgattctctgcttttgctagcaatatcctgtatgtagaaaagaaagcagaagtagattctctgttacccttcctgccctagggggattccacggatcctgagtcaccctgggagattatgaaactcaaaggtctttctcaaagatctttaaaaaccactgattctcaactgccaaattacagctactagtctttcctgatagtgttggctagacctcatggatgaccagaaggccttttcctcctctgcttctgtctaaaatgtcaggacttaggagcgcttgttatacatttcctggtaacagtaaattagaccgctatgactaagcgctagtgacagctgcgtagctaaagcaaaaccaaagccatcttctgtttgggttgcttagtttaatagaatagtgattgttttggctgggcacggtggctcacgcctgtaatcccagcactttgggaggccgaggtgggaggagtacttgagcccaggagttcgagaccagcctgggcaagatggtgaggccctatctctaccaaaaaaaaaaaaaaaaaaaaaaaaaaaaaaaaaaaaaaacttatcaaggaatccaaagaccttaccttcgaaaattgtaaaaaacagtaatacacaagcacatattcttttagtcaccagagcaatgacatcatcacatattctgtaaatgtataattatttcaaaaaaaagttaaaggaaatgaagcacagaagatgaatcaagtagggattacaacaactttcaacagcaaccgaagtcagaagacagataccatcaatgtgctgaaagaggaaaacttctgaacctcaaaatctataaactatgaaataaacccttcaagaattttaagatgggctggtccaaaggtagtgagttatctcagttgattgttcacaatcagttacacatcaaactccttattttactctgactactgcacttgactagtctaaaaaaagaattataagatgaattaaagacacgttcagataagcaaaactgagaacgtttggcaaaagcagatctttactaaaggaaattatgaagaatgtacctcgggcagaaggaaaagtgtcaagatcaagtgtcaaggaagattagagatttaagaaggtataagaaggttagaaaagtaagaaaaaaatatgccgtcaactctaaaaactacaagtataaagaaaaaagattattgggaaatccaaataacctaccttaggaaattctaaaagaatatacgagctcacattcctttggtcataagagcagtgtcatcattagacatcaggtcgcctctggaaaattccattgtgagtttaaaaggcaaatgacgtctataattctaaaactagttctcccaccgaaactctagaaaggatcttgggatctgcagggtctcccggatcacactttgagaactgctgctttagtcttcctcccatctcc

SEQ ID NO: 7 - DNA, 3743 bp, Artificial Sequence
  Synthetic: CCE7
acaggcactttccattaaccgaacaagctaaatgagctgtgccaagattctgaagcaataaaaatagatttaaattaccagggcgtggtgggggggggggcacctgtaatcccagctactcaggaagctgaggcagcagaatcgcttgaacccaggaggcagaggttgcagtgagccgagatcatgccactgcactccagcctgggcgacagagcaagactgtctcaaaaaaagaaaaaaatagatgtaagccatgtgcataatgtatagtacaccagaaatcacattctttgcaccttttttttttttttttgagacggagtttcactctgtcacccaggctggagtgcagtggtgtgatctcggctcactgcaacctccgcctcctgggttcaagcgattctcccgcctcagcctcccaaatagctgggattacaggtgcctgccaccacacccagctaattttttgtatttttagtagagacgggggtttcaccatgttggccaggctggtctcgaactccagacctcaggtgatcctcccgcctccgcctcccaaagcgctgggattacaggtgtgaaccaccgtgcccgacccctcagctctcagctcaatgtcgcttcctgcaatgtgtccattctacacagggaaatggcggaaggcagcaggtaaaaaaaatcacagcctttcctcatactgcttggcctttttttgttttttaaattctgaagaaagccatctccaagcacttccacctacatttcattggctgcaatgtgtcacctggcaacccttagctgtaagggagtctgggaattctagtattttgctttccagtttctctagtagaaaagtgtgtttctctagtaaaaagtgtttctcatgtgtgtaaagtgagcaaagtgataaagcatatattctaaaaagtaatttggggctgggtgcagcggctcttccctgtaatcctagcactttgggaggtcaaggtgagagggctgcttgaggccaggaatttgagactagtctgggcaacatagtaagactctgtctctacaaaaaattaagaaaatagctgggcatggtggcacatgcctgtagtcctagctacttgggaggctgaggcaggaagattccttgcacccaggagtttgaggctactattgttgccccactgcactccaacctgggtgacagagcaagaccctgtctttaaaaaaactaaataaataaatgaaaataaaaataaaaagtaggccaggtgcagcagcgcatgcctgtaatcccagcactttgggtggccaaggtgggaggatcgcttgagcccaggagttcgagaccagctttggcaacatggcaagaccccgtctcaatttaaaattttaaaaaccaataaaactaaaaagtaatttggaagactgtgaggtaaaccaaataatcaactaacaaagtagttacttaaaaaaacaaaacaagctgggcgtggtggctcatgcctctaatcccagcactttgggaggctgaggcaggcggatcacgaggtcaagagttcgagaccagcctggccaatatggtgaagcctcgtctctactaaaaatacaaaaattagctgggcatggtggcgcacacgtgtagtcccagctactcgggaggctgaggcagaagaatcgcttgaacccgagaggtggaggttgcagtgagccgagatcgtgccactgtgctccagcctgggcgacagagcgagacaccatctcaaaaataaaaataaaaataaataaaattaaaaaacaaaacaaggctaggctcagtggctcacgccagtaatcccagcactttgggtggtcaaagcaggaggattgcttgaggccaggagttcaagaccagcctgcacaacacagtgggaccctgtctctacaaaaataaataaataaataaatataaatataaatataaataaaaacaagccctccaaaaacctttgacagtgtgtaaagctatgcaattttctaatcgtgttaaagtaaaagcagttcacaaacaattcagactatacagaaataaaaagtagtatatatggcctaacattactttgttcttaaaattttccagtgacttttcttcccacttccaactccaactgccctattccagaatgtcaaatgattgtgacttgcaggttttctaatcagcacgtaagtcggaaattctaaaaatacattttaaattgtggatcacaccattacatgactgtctatagagccatttaattttgaaggcaagttaattttaaaaatagttacacacaaatgttcagttgattacgcttaagacagttttattctggtgattcagcatgatttttttcaacaaattaggtactttgtctgctttgtggaacattggcagtttcatttcctgttaaggaagctatcatcagaactcagataaacctttgcctttactatttgagtactgaaaataaacaaagaatataaaactcacatataggctgggtgcggtggctcacacgtgtaatcccagcactttgggaggccaaggcaggcggatcacttgaggccaggagtttgagaccagtccggccaacatggtaaaaccccatctctactaaaaatataaaaattagccaggcatggtggcacatacttgtaatcccacttacttgggaggctgaggcaggggaatcacttgagcccaggaggcagaagtagcagtgagccaaaatcatgccactgcactccagcctgggtgacagagcgagagtccgtctcaaaaaataaaataaaataaaaaataaaacacacgtatatacttggggacagaaacatcaaatatgttttctggatgatttaaaggtttagaaggggattatttattctaactgaaaaaaaaatcttttaatatgaattatttatatggaagacttctttttgaagctgttgtggctgatgctgttggattcatgtctaacttctttcattttataaaacagaatcatatcatcatcacaatctgtacactcccacctatactcttagggggcagtctggggtggttcctagggtaacaggcccaattatcccagtatacattgcatacagtaccctaacaacttttaggaaaggttttcattattagtgctttgttttagaaaaagtccaaaacaagccctaatgaagagtccaaaggataaggaagatgaagagaaagagaaagcactgaaaagtagaatcacatgatttgcaagtaggacaaggaaagcgagcaggaaaaaaaacagagttgtcagaacctgtggggaaaatgtgctgaacagcaagggctgagaaatgagcaacatattaaactttttttttttttttttttttttgagatggagtctcactgctgttgcccaggctggagtgcagtgccgacatctcagcttactgcaacctccatctcttgggttcaagtgaagctcctgcctcagccttctgagtagctgagattacaggcacccgccaccatgcccggctaattttttgtatttttagtagagacggtttcaccatgttggccaggaactcctgacgtcaggtgatccacccgcctcggcctcccaaagtgcccccatttcctttcattcgtttggagaactcctctactgcttgcatggttacctggtacaatgatcagtcatgatgccctgcccctctccaagaccatcccaaagagttggctcagg

SEQ ID NO: 8 - DNA, 3313 bp, Artificial Sequence
  Synthetic: CCE8
ccacagccagaacatgagaaattctttttttcccctcccagctcaatccttgtagaaaacaggaattctaaaggacaaataagccaggtttttcaacagataaatagcaagggacaatgagggagcggaaactattacagttctaagagacctatcagtcaaacacaacaggcagatcttgtttggatcctggttcaaacgaaccaactgtaaaaagttattcatgaaacaaccaggaaaatgtgtacattgaactggatattagatgatgttaaggaattagtgcaatttctttctttctttgagacggagtctctctctgttgcccaggctgggagtgtgcagtggcacgatcttggctcactgcaacctctacctcccgggttcaagcaattctcctgcctcagcctcctgagtagtttgaactacaggcatgagccaccatgcccggccttaatttcctttttttcttttttcttttttttttgagacagagtctcactctgtcacccaggctggagtgcagtggcgtgatctcggctcactgcaacctccgcctttcgggttcaagcgattcccctgcctcggcctcccgagtagctgggactacaggcgcacgccaccatgtctggctaatttttgtatttttagtagagacagggtttcaccatattggccaggctagtctcaaactcctaacctcatgatccgcccacctcagcttcccaaagtgctgggaccacaggcgtgagccaccacgcccagccccagcctaatttcttttttttttttttttccccaaatcaataggtcttttattgcatcatttaaatatcacaagtaggtcttaagtgtcatctggcatcttctttctgtagccaggtaactcttagatcttattcatcagcctgctgaacagttcctttttcagagacatagataccatccaaaaatttcctgatatccttgtttttaactgttgtggcttgctgaatcaaagccgctgaatttgaaacaagctcaatgtcatttccttcaaggattaattcatctttctgggcttgagatactgaacaagcaacacctggtctcatccgaaccctgcggatgtatttttcacccaaaaaatttcggatttcaacaagagacccattctcctggataacaacgttgatggggaagtgagcatacacagacctcatcttgtaacggaagcccagtgtaacacccttgatcatgttctgtacatgactacaaatagtccgaacggtagccagttcctttctgttaccccaccatttgtcaacccggagcctcttttttttctttccaagaaggctgagttctacattgatgtgattgaagtccctccgcagggttcctctggggcccttcacgataactgtgcgtcccttcagagtaatgtcgacattttctggaatgtcgacagtctgattgctgagaatagtcttcattctcgcagtagacgcagcaaagaaagcctaatttctttatgtatgataatataattacaattatatgccttcagtaagttttctgtgcagctactcagaagggtgaagtgggaggatcacctaaacccaggagttgaagtccagcctgggtaacacagcaagatcccatccccccagataaataacagtaaaaagaaagttttctgtgaacttgtaaaacaatatgtggaatatgatcccattttgtcaaaaaaccaaaaacatgcatgtatgcatgaatatattataaatgtataaataaatttatttaatttataaataaattttaaatataaataaatatatatatttgtttttgagacagggtatcactctgttgcccaggttggagtgcagtggagtgatcatggctcactgcaacctctttctcccaggctcaggagatcctcccacctcagcctccaagtaactgggactacaggtgttcgtcatcacactcagctaatttttttaattttttgtagagacagggtttcgccatattgcccaggctgttctcgaactgccagactcatataatccacctacctcagcctcccaaagtgctaggagtacaggtgtgagccactgcacccggcctatctatctatctatctatctatctatctatctatctatctatatttaaaagtctggaatgatataccaaactattaacaaaaattacctctggaaaaaagaataaaggggccagatgtggtggctcacacctgtaatcccagtactttgggaggctgaggcaggtggatcacctgaggtcaggagttcgagaccagcctgaccaatatgctaaaaccctgtctctactaaaaaatacaaaattagctgggcatggtggtgcatgcctgtaatcccagctacttgggaggctgaggcaggagaatgacttgaacccgggaggcctcagaggctgcagtgagcaagattgctccactgcactccagcctgggcaacaagagtgaaactctatctcaaaaaaaaaaaaaaaaaaaagaaagaaagaaaaagaaaagaataaaggataagacaagcttttttgttttgtttttgagacagagtttcactctttttgcccaggctagagtgcaatggcacgatctcggctcactgcaacctccgcctcctgggttcaagcgattctcctgcctcagcctcccaagtagctgggattacaggcaactaccaccatgcctggctttttttttttgtatttttagtagagacgggctttcaccatgttggccagggtggtctcgatctctcgacctcgtgatctgcccaccttggcctcccaaagtgctgggattacaggcgtgagccaccacacccggccaagacaagcttttaaaacagttagctaaaaacattttttacaaccaacacgaatcacttttataattaaaagctacacctcctccaataaagatctaaaaacaataaagaatgaagtcaaggttgtgtatttcagcaagctgaactctggtgcagagtatctttgaaaattgaaatggatatttacctaatttccctttattctatgtctttttcattgtccctgtacagaaatatatccattctggctgacagggatttaaaaaaagagagaaatataaccatattaaaagtcaagtctctagaggacatgtgtcactctgtggctgctcaccctccagtcatccttctaatggcacatcccatgcatatctggccccattcaccagagatactgattctggggtgccctttgccttttaccaagctccccgggtaatagtttg

SEQ ID NO: 9 - DNA, 3524 bp, Artificial Sequence
  Synthetic: CCE9
ggcgcgccccatcttcacatcatcatctcctctgtgtgtccgtcttataaggatacgtgtcattagatttaggactcacttgaatccagaatgatctcctcatcttaattatacttgcaaaagctcatcttccaaataaggtaacatccctaggctccgggaatcaggacgtagacgtatcttttgggagggcaccattcagcccactacacaggtcaaagttcattttttggtctatgtccagttgctccagcaccattcaaaaaggctatctttcttccattgaattgcttttgtacctttgttgaaaatcagtggggcatatttgtgtgggtctatttctaggttctctactctgtttcattgatctgtgtgtctgtccctccaccaatactacatagtcttgattattgtagctacataataagtcctgaaattggatagagtgattcctcccactttattctcccttttcaaaattgttttggctattctagtttctttgcctttccatataaattttggaataaacttgtctatgtttaaaatatcctcctggaattttgatagagattgagctaaaactatacataaatttggggagaactaacatctttactatgttaagtcttctgatccatgaatgtggcatatttctttctctatttaggtcttctttgatttctgtcatcagcattttgtagttttcagcatataagctctatacatatcttgttacatttacacttaagtattttgttcttgagcaagtgtaaatggcactgtatttttaatttcagcatccatgtgttcattgctagtatatagaaatacaatttatttttgcaagcttatcttgtatcctgcaaccttgctaagctcacttattagttctaggaattgtcttgtagattccttgggattttctatgtagactataatgccgtctccaaataggagcagttttatttattcttttataatctacatgttttatcttttcttttttcttctttttttttttttgccttattacactggttagaacttccaacactatgttgaattaaggtggtgagagcagagatccttgccttgtttccaatctgagggggaaagcatttagtctttcaagcattgtgtttaatgttaggtataagtctaatattgcttgatccagaaaaaaatatatatatatttggtgtaagttgtatgtagatgctcaagttaaggaagttccctttttgccctatttctcagagttttttttaacttataataagtgttagattttatcaaatgctttttctgcattgattaatatgatcatgtgatttctattagtttgttacactgattgtgtagaattagcatacaattctttaaacatttggtagaattctccagtgaaaccatctggacctggagattttaaagggagtagttttaaaattatgaatttcatgtttttaatagttatagggctattcaaatcatctatttcatatttggtagatttgggaagtttatatttttcaagaaattggtctgtttcatcaaagttgtcaaagcatgtagcattgttcatagtattcccttattacccatttgatgtctgaaggctctgtagtgatattcatttccttcctgatatgagcaatttgtatgtcttgctagaggtttgtcaatcttactgatcttttcaaagaagcagctctttatttcattgattttctctatttttctattttcaattctgcttatttatgctgttatttttattattttcttccttctgtttgctttggctttattttgctctccttgttctagttacttgaggtaggaacttagatgattgatttgagaccttttttcttttatagtataagcatttggagctataaacttctttttaagcattgctttagttgcatctcataaatttttctatgttgtattttcattttgattcagttcaatgtatttttaaaatttatcttgaaatttaaattttcatatttgacccatgggttattttaaagtgtgttgtttatttttcaagttttagatattttcttatctttctgttattgatttccaatttggtcacagaatacatttcatttgatttcaattattttaaatttgttgacatttgttttatgacacaggatatgtctaacatgttttgtattccatgggcacttgaaaaggatgtgtactcttctgctgttggatgagatgttctataaatgtcaaatcaaatcctgttgtttgagggtgttgttgagttcctatatacccttgctgattttctatctagtaggtctatcccagatgcctgctcagccttctctgacttcaccccagtggggaaatttggggcacctggttatagcttagcaagggtgaaaagctatgttttcaacccctcctttgctggtggggttgggaacgggaccacatatttttttctgtggtatttggctaaagaattagtgtataaaaatttctgtcttggtaagagagcatgatttttaaaaaatctgcccctgttggtattttcagtttgcagactttttcagcttcaactctgggatatatgaggcaaaacaaaaatccagggaactcaccacatgccgttccttgagtcctgaggtctcttgcaggtgtacattcttctctccacctcctctccagtctttttgtgttcattttatatataatgctcacggttttttgttgtgctttagagggaggaccagggaaaagtatgtcattccatcttcccagaagcagaagtcctaacttattcttttaaaatgttatgtaactttgcagagtatgacttttatcaggatttatttaactattcacccattgatgaacttttaggttgtttcttaattgtggtggctaacacaatctttcaataaacatccattcaataaacatttgtgtacacgtgcaggagtttcttcatgatagatgctaagtggcgttgctgggtaataggggatgcacattttccatgttaatgggtgttgtccaatttctacccataatggctgtgctccacccagcagtgtatgagagtagcagttttgctcaacttcttgacaacacttgataatagtcagactttgagttccgaatgtaatgagtgaaagatgatatctggtggttgttatcatttgcctttccttgattcccagaggctgaatatcttttcaaatgtctgttggccatctgtaactctccttttgaattacctgtccatatactttgcccatatttattttgagttgtttacctttttattgatttacagaaattctctatatatttttattgttctttgtctaatacatacatttcaaatatatttccccagtttattatttgtcttttaactttattgatggtgtcttttgcctaaaaaaaaattattcttttgtgtagattcaaatttgtcaaccactccctcctggcttttgggttgtgtttgtgtgttgacgcgt

SEQ ID NO: 10 - DNA, 3057 bp, Artificial Sequence
  Synthetic: CCE10
acgcgtcctccccttttccctagtttataagacaagagaaaagagagaaagcaaaaagttggaaagaaacaaaagtaagataaatagctagacgaccttggtgccaccacctggccctggtgattaaaataataatagtattaaccgctgaccaaaactactggtgctatctgtaaattccagacattgtatgagaaagcactgtaaaactttttgttctggccgggcgcggtggctcacgcctgtaatcccaggactttgggaggccgaggtgggaggatcatgaggtcaggagattgagaccatcctggctaacacggtgaaaccccatctctactaaaaatacaaaaaattagctgggtgcaggccgggcacggtggctccagcctctaatcccagcactttgggaggccgaggcgggtggatcacaaggtcaggagatcgagaccatcctggttaacatgatgaaaccccgtgtctactaaaaatacaaaaaattagccgggcgcggtggcgggcgcctgtagtcccagctactggggaggctgaggcaggagaatggtgtgaacccgggaggcggagcttgcagtgagctgagatcacgccactgcactccagcctgggccacagagcgagattccgtctcaaaaaaaataaaaaaataaaaactttttgttctcttagctgatgtatgtagcccccactcacgttcctcacacttacttgatctattatgactctttcacatagaccccttagagttcttagcccttaaaagggctaggaatttctttttcggggagctcggctcttaagacacgagtctgccgaatctcccggccaaataaaaaaacctcttccttctttaatctggtgtctgaggagttttgactgtgactcatcctgttacagcatgactggaaaaagaaaatgtggttcatccatataatgaaatatgaatcagccctaaaaaggaaggaatgatgagacaggctaccacatggactcacctgttgttaacaagataagccagacaaaaaagtgctgtgtgatcccactcctatgaggtctctggaagagtggaattcatagagacagacagtagaatggtgggtgccaggggccgggggaatggggcaccctggtttgatgtggacacagtttctgttttgtaagatgaagaagttgtaaacatctgttatacaacaatgcggatatgatgaacactgctgaagtgtatccttaaaaatactttaaaggggccgggcgcggtggctcatgcctgtaatcccagcactttgggaggccgaggcaggcggatcacgaggtcaggagatcgacaccgtcttggccaacacagtgaaaccccgtctctactaaaatacaaaaaatttgccaggtgtggtggcgggtgcctgtgatcccagctacttgggaggctgaggcaggggaatcacttgaacccgggaggtagaggttgaagtgagctgagattgtgccactgcactccagcctgggcaacagagcaagcctccatctaaaaaaaagaagtagttgaaagggtaaattttatgttatgtggcttttacctccattaaaaataaaaataaaggctgaatgtggtagcttacccctgtaatccgagcactttgggaggccaaagcaggacgattacttgagctcagaagtgtgagaccagcctggacaacttggtgagaccccatctctactagaaatttttttttaattggctgagtgtgatggtgtgcacctataatccccagatactcaggaggctgaggcaagaggattgcttgagcctaggagcggggggctgtggtgagccatgatggtaccattgcactccagcctgggtgacagagtgagaccctgcctcaaaaaaaaaaaaaaattaaattaagaaaaatttaaaaggccaggctaatgatatatttcttttattaataaacgtgggaaccttaatttaacataatgtcaataaacatgattatggttcttccaaatttggggtccctggtgagagaaaaagaataagatagggctgggtgtggtggtgcacgcctgtaatcccagcactttgggaggccaaggccagcagctcacctgaggttgggagttcgagaccagcctgaccaacatagagaatccccatctctaaaaatacaaaaaattagccaggcgtggtggcgcccacctgtaatcccagctacttgggaggctgaggccagagaattgcttgaacccgggaggcggaggttgcggtgagctgatatcacaccattgcactccagcctgggtaacaagagcgaaactccgtctctaataataataataataaataaagggcctcagggtgaagaatttggatactgcttgactggaggccacctggggccacttcagctctagtttctgtggtttacggccacagtggtgtcttccctgcaacgttctcgtgggtgccgtattgacaaaacattaaaacgagatggggtccctgcgagactcccgagggagggagcaggaagatccgtgcggcaccgcgaaggtacagcatgttctccacaactctcccaggccacaaagaaagatgagtcagtgggctctgaattctccagcacagacaggggacgagtcaaagggctcccaatcggacttgaagagatcacgcaggaagtcctgacgttcacggcgagcagggctctgtgtaggccaacatgccagcactgtgaggataatattttttaatcccccgtttccttgagcggccccagaaaacttacacacaccctgttctgcagactcctgggagtgtaggtctcattaagggcagatagagaccagactgtgcaacctttagaatctgcattgggcctaggtctcattgagggcaggtagagagccgactgtgcaacctttagagtctgcattgggccaaggtctcattgaggtcagatagagagcacactgtgcaacctttagagactgcattgagcctgggtctcattgaggacagatagagagcagaggcgcgcc

SEQ ID NO: 11 - DNA, 3313 bp, Artificial Sequence
  Synthetic: CCE11
ggcgcgccattttgggcagagattagttgggggatgtgggtgggaaacctggtgattagatatatttaaacgtgtcatgtcagtatagagcgtgaattaaaaataaattatatttggagagttgtaagaaatttaccagtcccttcagacagacacatgaccctttaaaactcattaaaactccttggcacaatggaataacatgcactttggtcttggaagaaaccattaggttgcaatgtttttgatttctctaccactgacttgctctttgatcttggaaagtgactgacttgtcctgtgattgtttcataatcacccataataaaactgacttactgtatatagtgaatagttaagtttaaaactatatctagtttccgttatagctcaagtttatgtattattttattagcgtttagatgttaacattaagctttcaaatcagatgaaatttaatttgaaaaaagttttcgtgtatgaatactttatattctgcagttcatacatgcagtaccacccttaattaaatgatatttccacaaatcagtttggaagattttcttcctgcaaaatgtatgtttaaaatacataaaaattgatgggaccatgtacttatggctagtcggaaagtggaaagttttttagatttatgcttaggacaggtgatagtacttgagcttctattcttagtttgaccttgcctcccccacccccttaaagcaagacacttaatctctttaatgtctcagtttattcatctttaacacctgtattcttatttcatgaaaacgatacctggtttatatttggtagcatttaaggacttgatatagaaggtggtatggaagttcaaattatatagaaagtatttgtatgctgaatgataatcttgacaaattactgattactacatttagaaagttacaactctggagggaattgatatttgatattgttttcctgtgtgttctaagttaccaccataacagtaggaaaataaaccctatcctggctgtgttacaaagggattaactcacttcttcaagttgttactaaatctccagccctttaaacaacagaaataaaaagtgttccttattttaatttttccgaaatgaaagtcctataactaaccttggcttaattttttcttttgttgagggctttccaagttattttctttgtgaggaatggaggctaaaccatgtcagttgcttgaagcaactaaaaataccccgtacaaatatgcagaggagtatgcttttgatttttagatcaaaacgaagaagcaagattttatggagcttgcttattatacatttattatactgagctacttgtgccttttcaaataattaaatattaactaaatacaagaggattaaatagctagactttaaataaaactaaaatagccatattagtattttctaaattctgtatcattgaaagtttaggctgatatgaaagagagggaattcctatcatggggattgccagtcttttcacaatgacctgccactagattttatagtatatgataaatgtgtgtgtgtttattgtgaaaattgtgtgagtcatatgaaaaattaagtctacttgaaaaatcaaaagacattacctacttgggtacaaagcctgatttatatatatatttctttaatgaccatattatgttatgttaaagtttgtatagtacttggacatatattatttaatttcattcctaaaacaattcaatagggaaagcaagacagatattaatattcccatttcatagatgaggaagaaaaaataacttggcttgtaagcaattcagcagagtcagagattgcatttgagatttttgattctaagtctagtgtgctttccttgggttacaacacaataaagtcaaaaacatttactgttattttcattaattgaaagcttaaaatcaatttaaaattctaacagtataaaatttaacagtataaaaatattgttaatttaattttatgacgttaatttttaaattgatttttgaatttgctaaaagtgttttaaaatcagtatcctgtttcacaattcctgaattaatctcttctctgtacatttcctgttccagtatgataatttatataggctttagcatttacttatggtattaaatgagtagacagttggaagggaattaaaattaattaggtcttgcagttcttataatactcctggtttgccacactgaattgccatgacgtggctggggatccctgttttaacatctaacaaagatagctgccagtgtacttaattttaaaacggtctcatctattaagctgctttataaacatcagccccttttctgaagtccaaagttagttttttaaaatattcactgataatggagtgggggtgctggtgacgtttctctttcttgtttatctgtaaagacagggaggtgcaatctaagttaggaaattggtgacaaatagtcatagaacatgggtcacctggcttcaattagttatgtgacctttaagaaaacaagtgcccgtttcagaaaagactgacctttgaggctagagacatcaagctactcctctacttttaggaaaaaacaatgacagggttaatttaaaactctgatgcagacagagttgaaaaatccatgacagatttatataacgaacgtggatggtgttttgttttcccagaatgcagttttaaggtcagacctatgactcagagctgtgcacttccctggtggtatgcatcagtgacatgttgccagtctaatcgtccagaagggcttgtgcccagctcggcttgctccattataatccccagctgagaagccacctttcattttttttaaatagataaggaagacagcatgaacatttgaaactcaaatactatatgtagtttataacttttcagcctgaagacttgatgcacactaagttgcctctttaattttgagaagtataatctccattgccactaatccatcatggtgtggcactgcatgaggatatgttgtgtgcattgtcagtatcggcgttttgctgagtttactgttttttagttcattggcaaggcatcgtgggttttggtgcaaagagcatggatttggaatcaaaagccacttcctctctgggtggctgattagctgagggtaaccttcacatagctggcatgggatttccagatggcatcctctctgcatgaacaaaaacaatgtgccatttcagtaaactttggtgggtgctccctcatccactccagatcttttcatctctttccttttattccctcccttacgcgt

SEQ ID NO: 12 - DNA, 3375 bp, Artificial Sequence
  Synthetic: CCE12
ccaacatggtgaaatctcatctccactaaacaaaaaaattatccagttgtggtggtgggcacctataatcccagctagtcgggaggctgaggcaggagagaatcgcttgaacccaggaggcagaggtagcagttagttgagatcatgccactgcactccagcctgggtgacagagtgagactctgcctccaaaaaaaaaaaaaaaatagactttagggaaaaaaaactataaaaagagatgaaaaatgtcattatatagtaataaaggagtaaatacatcaagagtatgtagcaattgtaaatttatatgtacccaacattatagcacttaaaataaatgtacagcaataattaagacattcaaagggagacaaagactgcagtgcaataataggaggaaacttcaatattccactttcaacattgaacagatcatccggggagaaaatcaataaggatacattgaacttgacctactttagaccaaatgaatataacagacatatgaaacatttaacccaacagcaacagaatacacattgttctcaatgcacatgatacattcttctggatagattatataataggccacaggccaggcacaatggctcatgcctgtaataacagcactttggaaggctgaggtgggaggatcatttgagcccagcccagaagttcaaggccagcctgggcaacatactgagaccctatctctaaaaacatgtatgtgtgtgtgtgtgcgtatatgtgtgtgtgtgtgtgtgtgtgtgtgtgtgtgtgtaataggtcacagaacaagtcttaacaaatttaagaagactgaaattatatcaagtatgttttccaaacacaatgttataaaactagaaatctgtaacataaagaaccatggaaaattggtggaatttgcggctttggcagattgaaataatggcaggtccagaaagtgatgcgcaataccagttcactggtattaaaaaatatttcaactcttatactctcacaggtagaatgaattgtgtactggtcacatacagaagcattgctttgattgtcttatatttcaagttaaggtccaaaaaaactccagctatgaaagcaacataaatggattttaaactgtctacagttcttaatctcatctgttaagttcccatgcctggagaagctaatgccaactcatcatgtgataattcaatttgtacaatatattatgaacttggaaaaaaaagaacatggaaaattaacaaatatgtgaaaattaaacaatatgctcctgagaaaatattaatattagagcaaagaagaaattaaagaagaaattttaaaatatcttgagactaacaaaaatggagacgcaacataccaaaacttaagagatgcagcaaaagcagttctaagaggaaattttatagcaataaatactaaaccaaaaaaaaaaaaaaaaggatctcaacaaaataacctaatgctacacctcaaggaactagaaaaagaagaacaaactaagcccaatgttagaagaagaaatgacaaaacaaaaatcagagcagaaataaatggattagagtctagaaaaacaatagaaaagatcaatgaaacagtatttttgcacgcattaaccaaattctctttatcccctccttccccactcccactcttcccagcttctggtaaccattaatttactcactatctccatgagatcacattttttagctcccacatatgaatgtgatcatgtgatatttgtctttctgtgcctggattatttcccttaacataatgtgactatagtttcaagcatgtattgtatatttcaaaacagctagactagaagatttggaatgtttccaacacaaaaaatgttaaatgtttcaggcaataattatctgaattaccctgatttgatcattatatattgtatgcatgtatcaaaatatcatatatacactatacatttgtacaatattatgtatcaattttaaaaatgtaagaaaagatcaatgaaactaaaagctagtatttggtagagctaaatgaaattgacaaactttagctagactaacaaaaagaaagaagactcaaataaataaactcatgaatgaaagaagggacattaaaactcaaaacacaaaaatacgaaggataatcagaaaaaactataaataattacacgtcaacaaagaggaaaacctagaaaaaatggataaatttctagaaacataaaacctaccaagactgaactaagaagaaattgattatctgaacagaccaataatgagtagggagattgaatcagtaataaagtctcctgtcaagaaaaaggtcaagaccagatggcttcatgactgaattccaccaaacatttaaataagaactaatactaatccttctcaaactcttccaaaaagttgaataggagaaaatacttccacactcattctatgaggccagcatcaccttgataccaaagccagacggacactacaaaaaagaaaaactctacaatgcagtatcactgataaacataaatgccaaattcctcaacaaatactagcaaaccatattcaacagtacattaaaaggataattcactgtgatcaagtgagatttatctcagggatgcaaggttggttcaacatattcaaatcagtaaatgtgattcaccatattaacagaataaaggacaaaaaccatatgatcatctccataaatgcagaaaaagaatttgacaaagttcaacattctttcatgataaaagctctcaacaaattaggtatagaaagactgttcctcaacacataaaggaaagccatatatgaccagcccacacctaacatcatactcaatggtgaaaagttaaaggcttttcctctaagagaaggaaaaaagacagatgcccactctcaccacttcttttcaacatagtaatagaagccctaaccagagcaattagacagaataaataaaaggcacccaaatagaaaatgataacgtgaaattgtctctgtttgctgacgacatgaatttatatatagaaaatcctgaagattttgccaaaactgctagaattgataaatgaattcagtataatcgcaggatacaaaatcaagttacaaaaattagtagcatttctatacactaacaatgaacgtaaaaagaaattaagaaaacaatcccatttataatagtatcaaaaaatacttaggagtaaatttaaccaaggaagtgaaatatctatatactgaaaactataaaactttgatgggaaaaaattaaagaggatgcaaacaaatggaaagataccttgtgttcatgaattataaaaattaatattgttaagacatccataatactctaggtgatgtacag

SEQ ID NO: 13 - DNA, 3000 bp, Artificial Sequence
  Synthetic: CCE13
tatatttgacttcactccatttcagcccttcctcacatcaacaagtaaaagtgaaagcaacgaggacctttttgggcttgtgccctttgaggaaataatggggagccagcagcaaaaagtcaaacagcgcagcttacagaaactgtcctctcgccaaaggcgcacaaagcaggatatgtccaaaagtaatgggaagcggcatcatggcacgccaactagcaaaaagaagactttgaagcctacctaccgcactccagagagggctcgcaggcacaaaaaagtgggtcgccgagtctctcaaaccagcaatgaatttgtaaccatctcagactccaaggagaacattggtgccgcagtgactgatgggaacgatagggggaacgtcttacaactcgaggagagtctgttggacccctttggtgccaagcccttccatcctccagacctgtcatggcaccctctacatcagggcctgaatgacatccgtgctgatcacaatactgtcctgcctaagcagccaaggcaaaattcactacatgggtcattccatagtgcagatgtattgacaatggatgattttggtgccatgccctttacagaacttgtggtgcaaagcatcactctacagcagtcccaacagtcccaaccagtcgaattagacccatttggtgctgccccatttccttctaaacagtagatacttctgatggattactggcattaactcctgtttcaaaaaagtatgaatagttttatgaatttgaaaaaaaatttaatggctgtttatgtcgttcgttcttaaagatcaatcagaacaggtgatttttaaaaaaccaaatagaaaaatgaagtatctctacagggtagtaacttgatgcctcttccaagcaggagaaaagggagctaaattgccagctctaactaagggtttctgctactgacctcacaacacagaaatgcaagtgtggtacttccagtgaaagcacatggcatccttccaggtgtgtaaccactcaggagggacagtaaaactgttatttttaatatcagaatgtcatttttgtgtgcatatccctaaaattagggttatttgtacatacactagttacgtttgtgaatttttttaagatctcttctaatttccatgcagttaaaaacaatctagttctcttaaagcattagaaagttattatctggagagtgcagagatttcactccatacacctttctccacaaagcagaaccagaagtaactggctattgtgcctaaaactatttcattttaaaaacaagtgccattaatatggaatatctaatgataagtacatgaaatgtatatattaatgtgtatattaattagctcaatttagctattccacaatttacatatttcaaaacaatgttatacatgataaatatatataatttttgtcaattaaaacataaattttaaaaatggactatcgcatagaagcctagaacaaaaatataaagagaaatatctgacattcaaaaagaaatgataagcagaaaaaataatatagaagaaaaaattcactactttagaaacactttatattgtttatgaatggcttcttgccccaaacttttattaacacggccctaatgaagcagattattggaaaaaattgggagtgaggacaagggttatataaaaattttattttaggaagaaaatatgtaggagaaactgaattttcaggacatttacagtgtgaaatcatgttgcatttaataatgtactttattagcaacttcaccaaatattccccaagtcataagcaacaattatttttattagttttggggggtggagtcgttttaataaagtgcacagaacagtgacatccacaaagccttataggcaggattcatgcatcctgctgcaagtacctctgcactaataaattagatcctaaaatgcatataaggtggactagcatcttaactctgctagttgatcatatcttcactgaaaagaacccagctaccaattgcctttttttaacaccacaaatgctaattagaaacttgagattttatagaaattatttaatgatagagattacatatgtgaattaatgtgaatatagtatctgtgcttcctgtgtctataaatattttaagttataattaactgtcctgcactatcagattaacatttcgaagtttctagaacagttaatgctatttacagaaaggagtggaaactcatcaactggcactctctttgatttttatattttaaattaactctctttgaacccaattaaagtatattttatgagtaattttgttaggcatctcttaattatagtgcctcaatgggataagatatttgcctattttcacagttctgaacttggaaagaagcaaagtatatgtaaataagccacatatttgtctttttattgcttttttccctcttttatatgctaaatcaaatataaatttgtggatagggaagcaatatgtgaatcacaatgtagcagaggcagaccaagcattacattattacttagagttgtacttttagagctggactgcaccaattacttgtcctcatgccaaaggcaaatatatttgcaacttttttttttcatttctcaggttgattaatactgctaatgcaaatgctcaagtagatgtttaaaaactttacaaaatagattcaaggaatactttcttttaaaagtgaagacttgatgattacacatagtaaattcatgaactacagtaggtttgtatcaaacagaataactttttaaatgaaaatcttttgaggtgtgcacaatatgcttcttattttagtccttggtctttgctagatctcatgagtttcatcatttagaaaaggggtaggggatgaactagtgtggtctccttcagatgtaaacatgaaatacctagcgttttactcgcttctcaatacactgaataattttaaatggttcagacactgatgtagaccctttggct

SEQ ID NO: 14 - DNA, 3556 bp, Artificial Sequence
  Synthetic: CCE14
cgaagagatttagaagaggggaaactcccaattacataaggtgggcattatagcttctcaaaacattggttccctatatgggtcatgaagattgatcccagtatcagcctatggcttactaggccagtttaactgaaagatttaatgagcttggaaggatgctgccacctgcactctcactttggcgggtgtttatcaccagtgagtgcggtccctaaaggagcaaaaggacaataagcacccagtggacaacagtgtggcattttgagtgaagatagcaactgaaaaggtcatcggcttggctagattgggctgggcttgttttttaaaaataaaaaaaaagttttccttcatgataaaagtaacaggtgatcattgttaaaaaataaagtatgaattaaaaagtaaataatatgtataattttataagccagaaaactaatttgtaatattcaggtgtatgtcctttcattctttttaaaaattatgtatataacacagttttataacaaaattgacatcatattgtatatatcattttattatctaattttttcatttgaaaattcacaagcatatttccatgttattgttctttgaaaaatacaatattaagtgctccataatatcttatggatttaacaaagtttatttagatgatgtcatgttattggacattttgattattaccaagtttgcgtataaaatttaaatgtaatgaacatcattgtacattaacctttatgcacatctggaattatttctttagaataaggttccagaattaaaattatttagtttggatgatgagagcatttattagagcatctgacaggtgatgctgaattttcctcaatacagttgtgcaaattgcattcccaccagtagtgtataaatgtgaatatccctccatatattcatcaaaacatggcctttctaattttgtaaatctctgctaatttaataggtaaaaatatacctttgttgctttaaaatttttatttctaatttacacacagtaaaattcactctttttagtatatggttctatgggttttgacaaatgcacagtcatgtatcttctacactagtaccatacagagaagttctgtcactttaataatttctcttggtggctctttttgtattcaaccccttaccccatactcaatctctggaaaccatcaatttattcttcatccctatggttttgccttttccagaaggtcatataagtggaatcaagcaatatgtagcccttttggtctggcttctttcacttagtaaaacgcagtcaagattctcccatgttttgtggataattatttcattcctttttatcactgagtagtacttcattgtgtggatgtaccacagttttattatccattcactaactgatgaacttgtaagatgtttctagttttggtgaatatgaacaaatttgctataaactttcaggtataagttttgtgtgataaatgctcatttttatagggtaaatgctttggagtgggaatgagtgccagactgttttctaaagtttccctagcattttgcattccaattacaaatatgtgagagttccagtagctttgtatctttaccagtatttagtaattttgtattatacatatatatgtatgtaaatatatatatatattcatttaaattttaatcattgttagaatttgtaattccccaatgatatatggtattatcttttatttgtttataattgacacataattatttatgggatacattgtgatgtttcagtacatgtgtacattgtataatgatcaaatcaggatatcacctcaaaccttatgatgatcttacagttaaagatgatatattcttgcaaagtgtctgttcagatcttttgctcccctttttattggattattccttttcttactgtttttatatgttttttaatatattgatacaaatcctttgtcagatacattatttggaaatagattttcctagtctgtgacttgtcttttcattctttgaacactgacttttttagagcaaaaattttaattttgatacaattcactttatcaatttttttacttttgatgtgcaatgtaagaacacttgtctaacccaatgtcatgaagattatatattattttcatccaggaattttatagttttaagttttacatttatatctatgatactttttgaataaaggtttgtataaagtttagctatgggtcaaggttcagtttttaaaatatggctatctaattgttctagtaccatttgttgaaaagattgtttcttttttattgcattgcttttgcacttctgtcaaaaaatcaattgattatatttgtttgggtctaattctgggctgcctattctgttccattgttatccattcacaaataccacactttcctaatcataggaagtcttaaaattagatagtgtgtacaacttcgtccgtctcaaaaatcgtgttgattactactttgcttttccagaaattttagaattgttgctttctataaaaaattctgctagtatatctgttgagttagaactatagatgaatttgaagaaaatttacatcctcacaatattttgtctttaggccacaaacatgatatagctgtatatttattttggtcttgcttttttttccactttcagcatacagatcctggacatattttatatttataccaaatattttatatattttctactgttgtcaatggtagtggtttttaaattttcaaacattcattactagtatatagaaataaaatcactttttaaaaatgtaatggcgtttattgtttttcaatttaataaaccacatttagacaacacaatgattaaaaatgttgacaattgggacgatgtaaatgtaaaggtaaaggtaacaatttttaccttgataatataaaggtaaaaatgtagtagacagtatatggggacagaagaggaagtgtgtaggaagggcagagtgggaatattaatagcatcatcttttatagagagaacacactgatgtgattgaacaccaaataggggtatatgcatctgaaagtcacttttggtatgttgaccttgtatcctgcaactttgctaaactcatttattatatgaacttttatgtatatttcttggcattttctacatacagtggtgtctgtatagtttactatttacatgtgaatatggatagtttaatttcttcctttccaatttgcttgccttttatgtcttcttgaaatactgcgttggctaagacttgcagtaagaagttaaaagggaatgtttggagcacacgtatttgccaagtctctgatcttagtgtggctggggggaagcatttagtatttcattaagtatgatgttagctataggttttttgtagatattctttatcagtttaagaaaatttcctatgattactagattgttcagaattgttttaagatcatgagttgatatttcaattttgttaaatactttttctgtatccattaagataatcatgtgtttttcttagtcagtcattgtagcc

SEQ ID NO: 15 - DNA, 913 bp, Artificial Sequence
  Synthetic: core CCE14 #7
cgaagagatttagaagaggggaaactcccaattacataaggtgggcattatagcttctcaaaacattggttccctatatgggtcatgaagattgatcccagtatcagcctatggcttactaggccagtttaactgaaagatttaatgagcttggaaggatgctgccacctgcactctcactttggcgggtgtttatcaccagtgagtgcggtccctaaaggagcaaaaggacaataagcacccagtggacaacagtgtggcattttgagtgaagatagcaactgaaaaggtcatcggcttggctagattgggctgggcttgttttttaaaaataaaaaaaaagttttccttcatgataaaagtaacaggtgatcattgttaaaaaataaagtatgaattaaaaagtaaataatatgtataattttataagccagaaaactaatttgtaatattcaggtgtatgtcctttcattctttttaaaaattatgtatataacacagttttataacaaaattgacatcatattgtatatatcattttattatctaattttttcatttgaaaattcacaagcatatttccatgttattgttctttgaaaaatacaatattaagtgctccataatatcttatggatttaacaaagtttatttagatgatgtcatgttattggacattttgattattaccaagtttgcgtataaaatttaaatgtaatgaacatcattgtacattaacctttatgcacatctggaattatttctttagaataaggttccagaattaaaattatttagtttggatgatgagagcatttattagagcatctgacaggtgatgctgaattttcctcaatacagttgtgcaaattgcattcccaccagtagtgtataaatgtgaatatccctccat

SEQ ID NO: 16 - DNA, 1405 bp, Artificial Sequence
  Synthetic: core CCE14 #8
cgaagagatttagaagaggggaaactcccaattacataaggtgggcattatagcttctcaaaacattggttccctatatgggtcatgaagattgatcccagtatcagcctatggcttactaggccagtttaactgaaagatttaatgagcttggaaggatgctgccacctgcactctcactttggcgggtgtttatcaccagtgagtgcggtccctaaaggagcaaaaggacaataagcacccagtggacaacagtgtggcattttgagtgaagatagcaactgaaaaggtcatcggcttggctagattgggctgggcttgttttttaaaaataaaaaaaaagttttccttcatgataaaagtaacaggtgatcattgttaaaaaataaagtatgaattaaaaagtaaataatatgtataattttataagccagaaaactaatttgtaatattcaggtgtatgtcctttcattctttttaaaaattatgtatataacacagttttataacaaaattgacatcatattgtatatatcattttattatctaattttttcatttgaaaattcacaagcatatttccatgttattgttctttgaaaaatacaatattaagtgctccataatatcttatggatttaacaaagtttatttagatgatgtcatgttattggacattttgattattaccaagtttgcgtataaaatttaaatgtaatgaacatcattgtacattaacctttatgcacatctggaattatttctttagaataaggttccagaattaaaattatttagtttggatgatgagagcatttattagagcatctgacaggtgatgctgaattttcctcaatacagttgtgcaaattgcattcccaccagtagtgtataaatgtgaatatccctccatatattcatcaaaacatggcctttctaattttgtaaatctctgctaatttaataggtaaaaatatacctttgttgctttaaaatttttatttctaatttacacacagtaaaattcactctttttagtatatggttctatgggttttgacaaatgcacagtcatgtatcttctacactagtaccatacagagaagttctgtcactttaataatttctcttggtggctctttttgtattcaaccccttaccccatactcaatctctggaaaccatcaatttattcttcatccctatggttttgccttttccagaaggtcatataagtggaatcaagcaatatgtagcccttttggtctggcttctttcacttagtaaaacgcagtcaagattctcccatgttttgtggataattatttcattcctttttatcactgagtagtacttcattgtgtggatgtaccacagttttattatccattcactaactgatgaa

SEQ ID NO: 17 - DNA, 32 bp, Artificial Sequence
  Synthetic: CCE1_F primer
agaaggcgcgcgactgtggactccaggaagct

SEQ ID NO: 18 - DNA, 31 bp, Artificial Sequence
  Synthetic: CCE1_R primer
agaaacgcgtgatgtaacccacagaacactg

SEQ ID NO: 19 - DNA, 34 bp, Artificial Sequence
  Synthetic: CCE2-P139 primer
agaaggcgcgccttgtgtgggtctatttctaggt

SEQ ID NO: 20 - DNA, 32 bp, Artificial Sequence
  Synthetic: CCE2-P144 primer
agaaacgcgtgtggagaaaaggagaaaagatg

SEQ ID NO: 21 - DNA, 32 bp, Artificial Sequence
  Synthetic: CCE2-P134 primer
agaaacgcgtttgtgtgggtctatttctaggt

SEQ ID NO: 22 - DNA, 34 bp, Artificial Sequence
  Synthetic: CCE2-P149 primer
agaaggcgcgccgtggagaaaaggagaaaagatg

SEQ ID NO: 23 - DNA, 34 bp, Artificial Sequence
  Synthetic: CCE3-F primer
agaaggcgcgccggctattctttctttccgcatt

SEQ ID NO: 24 - DNA, 32 bp, Artificial Sequence
  Synthetic: CCE3-R primer
agaaacgcgttgtattttttgtaagggggggg

SEQ ID NO: 25 - DNA, 32 bp, Artificial Sequence
  Synthetic: CCE4-F primer
agaaacgcgtttttgggcagagattagttggg

SEQ ID NO: 26 - DNA, 34 bp, Artificial Sequence
  Synthetic: CCE4-R primer
agaaggcgcgccaagggagggaataaaaggaaag

SEQ ID NO: 27 - DNA, 32 bp, Artificial Sequence
  Synthetic: CCE5-F primer
agaaacgcgttgctgttgttggatgaggtagt

SEQ ID NO: 28 - DNA, 32 bp, Artificial Sequence
  Synthetic: CCE5-R primer
agaaacgcgtggatattggtttagctgctggt

SEQ ID NO: 29 - DNA, 32 bp, Artificial Sequence
  Synthetic: CCE6-F primer
agaaggcgcgcccgtctgttttgtttcggttt

SEQ ID NO: 30 - DNA, 31 bp, Artificial Sequence
  Synthetic: CCE6-R primer
agaaacgcgtggagatgggaggaagactaaa

SEQ ID NO: 31 - DNA, 33 bp, Artificial Sequence
  Synthetic: CCE7-F primer
agaaggcgcgccacaggcactttccattaaccg

SEQ ID NO: 32 - DNA, 30 bp, Artificial Sequence
  Synthetic: CCE7-R primer
agaaacgcgtcctgagccaactctttggga

SEQ ID NO: 33 - DNA, 30 bp, Artificial Sequence
  Synthetic: CCE8-F primer
agaaacgcgtccacagccagaacatgagaa

SEQ ID NO: 34 - DNA, 30 bp, Artificial Sequence
  Synthetic: CCE8-R primer
agaaacgcgtcaaactattacccggggagc

SEQ ID NO: 35 - DNA, 34 bp, Artificial Sequence
  Synthetic: CCE9-F primer
agaaggcgcgccccatcttcacatcatcatctcc

SEQ ID NO: 36 - DNA, 32 bp, Artificial Sequence
  Synthetic: CCE9-R primer
agaaacgcgtcaacacacaaacacaacccaaa

SEQ ID NO: 37 - DNA, 34 bp, Artificial Sequence
  Synthetic: CCE10-P262 primer
agaaggcgcgcccctccccttttccctagtttat

SEQ ID NO: 38 - DNA, 32 bp, Artificial Sequence
  Synthetic: CCE10-P267 primer
agaaacgcgttctgctctctatctgtcctcaa

SEQ ID NO: 39 - DNA, 31 bp, Artificial Sequence
  Synthetic: CCE10-P257 primer
agaaacgcgcctccccttttccctagtttat

SEQ ID NO: 40 - DNA, 34 bp, Artificial Sequence
  Synthetic: CCE10-P272 primer
agaaggcgcgcctctgctctctatctgtcctcaa

SEQ ID NO: 41 - DNA, 34 bp, Artificial Sequence
  Synthetic: CCE11-F primer
agaaggcgcgccattttgggcagagattagttgg

SEQ ID NO: 42 - DNA, 32 bp, Artificial Sequence
  Synthetic: CCE11-R primer
agaaacgcgtaagggagggaataaaaggaaag

SEQ ID NO: 43 - DNA, 34 bp, Artificial Sequence
  Synthetic: CCE12-F primer
agaaggcgcgccgggctacaatgactgactaaga

SEQ ID NO: 44 - DNA, 32 bp, Artificial Sequence
  Synthetic: CCE12-R primer
agaaacgcgtgaagagatttagaagaggggaa

SEQ ID NO: 45 - DNA, 32 bp, Artificial Sequence
  Synthetic: CCE13-F primer
aaggcgcgcccacgccaactagcacaaagaag

SEQ ID NO: 46 - DNA, 36 bp, Artificial Sequence
  Synthetic: CCE13-P127 primer
agaaggcgcgcctctgggggatgatgaatgaaaatg

SEQ ID NO: 47 - DNA, 35 bp, Artificial Sequence
  Synthetic: CCE14-F primer
aaggcgcgcccaacatggtgaaatctcatctccac

SEQ ID NO: 48 - DNA, 38 bp, Artificial Sequence
  Synthetic: CCE14-R primer
aaacgcgtctgtacatcacctagagtattatggatgtc